European Patent Specification EP 4 240 396 B1, published January 1, 2025. Title: Use of IFN-Lambda mRNA for treating viral infections. Applicant: ethris GmbH. The sequence listing filed with the application follows.

SEQUENCE LISTING (36 sequences)

SEQ ID NO: 1 - RNA, 603 nt, Homo sapiens
  IFN Lambda 1
  CDS 1..603: /transl_table=1
auggcugcugcuuggacaguggugcuggucacacuggugcugggacuugcuguggcuggaccugugccuaccagcaagccuaccacaacaggcaagggcugccacaucggcagauucaagagccugucuccucaagagcuggccuccuucaagaaagccagggacgcccuggaagagagccugaagcugaagaacugguccugcagcagcccuguguuccccggcaauugggaucugagacugcugcaagugcgcgagaggccuguugcucuggaagcugaacuggcccugacacugaaggugcuggaagccgcugcuggacccgcacuggaagauguucuggaucagccucugcacacccugcaccacauucugagucagcugcaggccuguauccagccucagccuacagcuggcccuagaccuagaggcagacugcaccacuggcugcacagacugcaagaggccccuaagaaagagagcgccggcugucuggaagccagcgugaccuucaaccuguucagacugcugacccgggaccugaaauacguggccgauggcaaucugugccugcggacaucuacacaccccgagagcacauga

SEQ ID NO: 2 - protein, 200 aa, Homo sapiens
  [CDS]:1..603 from SEQ ID NO 1
MAAAWTVVLVTLVLGLAVAGPVPTSKPTTTGKGCHIGRFKSLSPQELASFKKARDALEESLKLKNWSCSSPVFPGNWDLRLLQVRERPVALEAELALTLKVLEAAAGPALEDVLDQPLHTLHHILSQLQACIQPQPTAGPRPRGRLHHWLHRLQEAPKKESAGCLEASVTFNLFRLLTRDLKYVADGNLCLRTSTHPEST

SEQ ID NO: 3 - RNA, 603 nt, Homo sapiens
  IFN Lambda 2
  CDS 1..603: /transl_table=1
augaagcuggacaugaccggcgauugcaccccugugcugguucugauggcugccgugcugacagugacaggugcugugccuguggcuagacugcauggcgcacugccugaugccagaggcugucacauugcccaguucaagagccugucuccucaagagcugcaggccuucaagagagccaaggacgcccuggaagagagccugcugcugaaggauugccggugccacagcagacuguuccccagaaccugggaccugagacagcugcaagugcgcgaaagacccauggcucuggaagccgaacuggcccugacacugaaagugcuggaagccaccgccgacaccgauccugcucugguggauguucuggaccagccucugcacacccugcaccacauccugagccaguucagggccuguauccagccucagccuacagcuggcccuagaaccagaggcagacugcaccacuggcuguacagacugcaagaggccccuaagaaagagagccccggcugucuggaagcuagcgugaccuucaaccuguuccggcugcugaccagggaccugaauuguguggcuagcggcgaccugugcguguga

SEQ ID NO: 4 - protein, 200 aa, Homo sapiens
  [CDS]:1..603 from SEQ ID NO 3
MKLDMTGDCTPVLVLMAAVLTVTGAVPVARLHGALPDARGCHIAQFKSLSPQELQAFKRAKDALEESLLLKDCRCHSRLFPRTWDLRQLQVRERPMALEAELALTLKVLEATADTDPALVDVLDQPLHTLHHILSQFRACIQPQPTAGPRTRGRLHHWLYRLQEAPKKESPGCLEASVTFNLFRLLTRDLNCVASGDLCV

SEQ ID NO: 5 - RNA, 591 nt, Homo sapiens
  IFN Lambda 3
  CDS 1..591: /transl_table=1
augacaggcgauugcaugccugugcuggugcugauggcugccgugcugacaguuacaggugcugugccuguggccagacugagaggugcacugccugaugccagaggcugucacauugcccaguucaagagccugucuccucaagagcugcaggccuucaagagagccaaggacgcccuggaagagagccugcugcugaaggacugcaagugcagaagccggcuguuccccagaaccugggaucugagacagcugcaaguccgcgaaagacccguggcucuggaagcugaacuggcccugacacugaaggugcuggaagccaccgccgauaccgauccugcucugggagaugugcuggaccagccucugcacacacugcaccacauccugagccagcugagggccuguauucagccccaaccuacagcuggcccucggacaagaggcagacugcaccauuggcugcaccggcugcaagaggccccuaagaaagagucuccuggcugccuggaagccuccgugaccuucaaccuguucagacugcugacccgggaccugaauuguguggccucuggcgaucugugcguguga

SEQ ID NO: 6 - protein, 196 aa, Homo sapiens
  [CDS]:1..591 from SEQ ID NO 5
MTGDCMPVLVLMAAVLTVTGAVPVARLRGALPDARGCHIAQFKSLSPQELQAFKRAKDALEESLLLKDCKCRSRLFPRTWDLRQLQVRERPVALEAELALTLKVLEATADTDPALGDVLDQPLHTLHHILSQLRACIQPQPTAGPRTRGRLHHWLHRLQEAPKKESPGCLEASVTFNLFRLLTRDLNCVASGDLCV

SEQ ID NO: 7 - DNA, 13 bp, Artificial Sequence
  primer
gggagacgccacc

SEQ ID NO: 8 - DNA, 17 bp, Artificial Sequence
  primer
taatacgactcactata

SEQ ID NO: 9 - DNA, 30 bp, Artificial Sequence
  primer
taatacgactcactatagggagacgccacc

SEQ ID NO: 10 - DNA, 637 bp, Homo sapiens
  DNA construct IFN Lambda 1
taatacgactcactatagggagacgccaccatggctgctgcttggacagtggtgctggtcacactggtgctgggacttgctgtggctggacctgtgcctaccagcaagcctaccacaacaggcaagggctgccacatcggcagattcaagagcctgtctcctcaagagctggcctccttcaagaaagccagggacgccctggaagagagcctgaagctgaagaactggtcctgcagcagccctgtgttccccggcaattgggatctgagactgctgcaagtgcgcgagaggcctgttgctctggaagctgaactggccctgacactgaaggtgctggaagccgctgctggacccgcactggaagatgttctggatcagcctctgcacaccctgcaccacattctgagtcagctgcaggcctgtatccagcctcagcctacagctggccctagacctagaggcagactgcaccactggctgcacagactgcaagaggcccctaagaaagagagcgccggctgtctggaagccagcgtgaccttcaacctgttcagactgctgacccgggacctgaaatacgtggccgatggcaatctgtgcctgcggacatctacacaccccgagagcacatgattcg

SEQ ID NO: 11 - DNA, 637 bp, Homo sapiens
  DNA construct IFN Lambda 2
taatacgactcactatagggagacgccaccatgaagctggacatgaccggcgattgcacccctgtgctggttctgatggctgccgtgctgacagtgacaggtgctgtgcctgtggctagactgcatggcgcactgcctgatgccagaggctgtcacattgcccagttcaagagcctgtctcctcaagagctgcaggccttcaagagagccaaggacgccctggaagagagcctgctgctgaaggattgccggtgccacagcagactgttccccagaacctgggacctgagacagctgcaagtgcgcgaaagacccatggctctggaagccgaactggccctgacactgaaagtgctggaagccaccgccgacaccgatcctgctctggtggatgttctggaccagcctctgcacaccctgcaccacatcctgagccagttcagggcctgtatccagcctcagcctacagctggccctagaaccagaggcagactgcaccactggctgtacagactgcaagaggcccctaagaaagagagccccggctgtctggaagctagcgtgaccttcaacctgttccggctgctgaccagggacctgaattgtgtggctagcggcgacctgtgcgtgtgattcg

SEQ ID NO: 12 - DNA, 625 bp, Homo sapiens
  DNA construct IFN Lambda 3
taatacgactcactatagggagacgccaccatgacaggcgattgcatgcctgtgctggtgctgatggctgccgtgctgacagttacaggtgctgtgcctgtggccagactgagaggtgcactgcctgatgccagaggctgtcacattgcccagttcaagagcctgtctcctcaagagctgcaggccttcaagagagccaaggacgccctggaagagagcctgctgctgaaggactgcaagtgcagaagccggctgttccccagaacctgggatctgagacagctgcaagtccgcgaaagacccgtggctctggaagctgaactggccctgacactgaaggtgctggaagccaccgccgataccgatcctgctctgggagatgtgctggaccagcctctgcacacactgcaccacatcctgagccagctgagggcctgtattcagccccaacctacagctggccctcggacaagaggcagactgcaccattggctgcaccggctgcaagaggcccctaagaaagagtctcctggctgcctggaagcctccgtgaccttcaacctgttcagactgctgacccgggacctgaattgtgtggcctctggcgatctgtgcgtgtgattcg

SEQ ID NO: 13 - RNA, 620 nt, Homo sapiens
  mRNA construct for IFN Lambda 1
gggagacgccaccauggcugcugcuuggacaguggugcuggucacacuggugcugggacuugcuguggcuggaccugugccuaccagcaagccuaccacaacaggcaagggcugccacaucggcagauucaagagccugucuccucaagagcuggccuccuucaagaaagccagggacgcccuggaagagagccugaagcugaagaacugguccugcagcagcccuguguuccccggcaauugggaucugagacugcugcaagugcgcgagaggccuguugcucuggaagcugaacuggcccugacacugaaggugcuggaagccgcugcuggacccgcacuggaagauguucuggaucagccucugcacacccugcaccacauucugagucagcugcaggccuguauccagccucagccuacagcuggcccuagaccuagaggcagacugcaccacuggcugcacagacugcaagaggccccuaagaaagagagcgccggcugucuggaagccagcgugaccuucaaccuguucagacugcugacccgggaccugaaauacguggccgauggcaaucugugccugcggacaucuacacaccccgagagcacaugauucg

SEQ ID NO: 14 - RNA, 620 nt, Homo sapiens
  mRNA construct for IFN Lambda 2
gggagacgccaccaugaagcuggacaugaccggcgauugcaccccugugcugguucugauggcugccgugcugacagugacaggugcugugccuguggcuagacugcauggcgcacugccugaugccagaggcugucacauugcccaguucaagagccugucuccucaagagcugcaggccuucaagagagccaaggacgcccuggaagagagccugcugcugaaggauugccggugccacagcagacuguuccccagaaccugggaccugagacagcugcaagugcgcgaaagacccauggcucuggaagccgaacuggcccugacacugaaagugcuggaagccaccgccgacaccgauccugcucugguggauguucuggaccagccucugcacacccugcaccacauccugagccaguucagggccuguauccagccucagccuacagcuggcccuagaaccagaggcagacugcaccacuggcuguacagacugcaagaggccccuaagaaagagagccccggcugucuggaagcuagcgugaccuucaaccuguuccggcugcugaccagggaccugaauuguguggcuagcggcgaccugugcgugugauucg

SEQ ID NO: 15 - RNA, 597 nt, Homo sapiens
  mRNA construct for IFN Lambda 3
gggagacgccaccaugacaggcgauugcaugccugugcuggugcugauggcugccgugcugacaguuacaggugcugugccuguggccagacugagaggugcacugccugaugccagaggcugucacauugcccaguucaagagccugucuccucaagagcugcaggccuucaagagagccaaggacgcccuggaagagagccugcugcugaaggacugcaagugcagaagccggcuguuccccagaaccugggaucugagacagcugcaaguccgcgaaagacccguggcucuggaagcugaacuggcccugacacugaaggugcuggaagccaccgccgauaccgauccugcucugggagaugugcuggaccagccucugcacacacugcaccacauccugagccagcugagggccuguauucagccccaaccuacagcuggcccucggacaagaggcagacugcaccauuggcugcaccggcugcaagaggccccuaagaaagagucuccuggcugccuggaagccuccgugaccuucaaccuguucagacugcugacccgggaccugaauuguguggccucuggcgaucugug

SEQ ID NO: 16 - RNA, 570 nt, Homo sapiens
  IFN alpha 16
  CDS 1..570: /transl_table=1
auggcccugagcuucucucugcugauggcugugcuggugcugagcuacaagagcaucugcagccugggcugcgaccugccucagacacacucucugggaaacagacgggcccugauucugcuggcccagaugggcagaaucucccacuucagcugccugaaggacagauacgacuucggcuucccucaagagguguucgacggcaaccaguuccagaaggcccaggccaucucugccuuccacgagaugauccagcagaccuucaaccuguucagcaccaaggauagcagcgccgccugggaugagacacugcuggacaaguucuacaucgagcuguuccagcagcugaacgaccuggaagccugcgugacacaagaagugggcgucgaagagaucgcccugaugaacgaggauagcauccuggccgugcgcaaguacuuccagcggaucacccuguaccugaugggcaagaaguacagcccuugcgccugggaagucgugcgggccgaaaucaugagaagcuucagcuuuagcaccaaccugcagaagggccugagaagaaaggacuga

SEQ ID NO: 17 - protein, 189 aa, Homo sapiens
  [CDS]:1..570 from SEQ ID NO 16
MALSFSLLMAVLVLSYKSICSLGCDLPQTHSLGNRRALILLAQMGRISHFSCLKDRYDFGFPQEVFDGNQFQKAQAISAFHEMIQQTFNLFSTKDSSAAWDETLLDKFYIELFQQLNDLEACVTQEVGVEEIALMNEDSILAVRKYFQRITLYLMGKKYSPCAWEVVRAEIMRSFSFSTNLQKGLRRKD

SEQ ID NO: 18 - RNA, 564 nt, Homo sapiens
  IFN beta
  CDS 1..564: /transl_table=1
augaccaacaagugccugcugcagauugcccugcugcugugcuucagcacaacagcccugagcaugagcuacaaccugcugggcuuccugcagcggagcagcaacuuccagugccagaaacugcuguggcagcugaacggccggcuggaauacugccugaaggaccggaugaacuucgacauccccgaggaaaucaagcagcugcagcaguuccagaaagaggacgccgcucugaccaucuacgagaugcugcagaacaucuucgccaucuuccggcaggacagcagcuccacaggcuggaacgagacaaucguggaaaaucugcuggccaacguguaccaccagaucaaccaccugaaaaccgugcuggaagagaagcuggaaaaagaggacuucacccggggcaagcugaugagcagccugcaccugaagcgguacuacggcagaauccugcacuaccugaaggccaaagaguacagccacugcgccuggaccaucgugcgcguggaaauccugcggaacuucuacuucaucaaccggcugaccggcuaccugagaaacuga

SEQ ID NO: 19 - protein, 187 aa, Homo sapiens
  [CDS]:1..564 from SEQ ID NO 18
MTNKCLLQIALLLCFSTTALSMSYNLLGFLQRSSNFQCQKLLWQLNGRLEYCLKDRMNFDIPEEIKQLQQFQKEDAALTIYEMLQNIFAIFRQDSSSTGWNETIVENLLANVYHQINHLKTVLEEKLEKEDFTRGKLMSSLHLKRYYGRILHYLKAKEYSHCAWTIVRVEILRNFYFINRLTGYLRN

SEQ ID NO: 20 - RNA, 501 nt, Homo sapiens
  IFN gamma
  CDS 1..501: /transl_table=1
augaaguacaccagcuacauccuggccuuccagcugugcaucgugcugggaagccugggcugcuacugccaggauccuuacgugaaagaggccgagaaccugaagaaguacuuuaacgccggccacagcgacguggccgacaauggaacacuguuccugggcauccugaagaacuggaaagaggaaagcgaccggaagaucaugcagagccagaucguguccuucuacuucaagcuguucaagaacuucaaggacgaccagagcauccagaaaagcguggaaaccaucaaagaagauaugaacgucaaguucuucaacuccaacaagaagaagcgggacgacuucgagaagcugaccaacuacagcgugaccgaccugaacgugcagagaaaggccauccacgagcugauccaagugauggccgaacugucuccugccgccaagaccggaaagcggaagagaagccagaugcuguucagaggcagacgggccucucaguga

SEQ ID NO: 21 - protein, 166 aa, Homo sapiens
  [CDS]:1..501 from SEQ ID NO 20
MKYTSYILAFQLCIVLGSLGCYCQDPYVKEAENLKKYFNAGHSDVADNGTLFLGILKNWKEESDRKIMQSQIVSFYFKLFKNFKDDQSIQKSVETIKEDMNVKFFNSNKKKRDDFEKLTNYSVTDLNVQRKAIHELIQVMAELSPAAKTGKRKRSQMLFRGRRASQ

SEQ ID NO: 22 - DNA, 604 bp, Homo sapiens
  DNA construct IFN alpha 16
taatacgactcactatagggagacgccaccatggccctgagcttctctctgctgatggctgtgctggtgctgagctacaagagcatctgcagcctgggctgcgacctgcctcagacacactctctgggaaacagacgggccctgattctgctggcccagatgggcagaatctcccacttcagctgcctgaaggacagatacgacttcggcttccctcaagaggtgttcgacggcaaccagttccagaaggcccaggccatctctgccttccacgagatgatccagcagaccttcaacctgttcagcaccaaggatagcagcgccgcctgggatgagacactgctggacaagttctacatcgagctgttccagcagctgaacgacctggaagcctgcgtgacacaagaagtgggcgtcgaagagatcgccctgatgaacgaggatagcatcctggccgtgcgcaagtacttccagcggatcaccctgtacctgatgggcaagaagtacagcccttgcgcctgggaagtcgtgcgggccgaaatcatgagaagcttcagctttagcaccaacctgcagaagggcctgagaagaaaggactgattcg

SEQ ID NO: 23 - DNA, 598 bp, Homo sapiens
  DNA construct IFN beta
taatacgactcactatagggagacgccaccatgaccaacaagtgcctgctgcagattgccctgctgctgtgcttcagcacaacagccctgagcatgagctacaacctgctgggcttcctgcagcggagcagcaacttccagtgccagaaactgctgtggcagctgaacggccggctggaatactgcctgaaggaccggatgaacttcgacatccccgaggaaatcaagcagctgcagcagttccagaaagaggacgccgctctgaccatctacgagatgctgcagaacatcttcgccatcttccggcaggacagcagctccacaggctggaacgagacaatcgtggaaaatctgctggccaacgtgtaccaccagatcaaccacctgaaaaccgtgctggaagagaagctggaaaaagaggacttcacccggggcaagctgatgagcagcctgcacctgaagcggtactacggcagaatcctgcactacctgaaggccaaagagtacagccactgcgcctggaccatcgtgcgcgtggaaatcctgcggaacttctacttcatcaaccggctgaccggctacctgagaaactgattcg

SEQ ID NO: 24 - DNA, 535 bp, Homo sapiens
  DNA construct IFN gamma
taatacgactcactatagggagacgccaccatgaagtacaccagctacatcctggccttccagctgtgcatcgtgctgggaagcctgggctgctactgccaggatccttacgtgaaagaggccgagaacctgaagaagtactttaacgccggccacagcgacgtggccgacaatggaacactgttcctgggcatcctgaagaactggaaagaggaaagcgaccggaagatcatgcagagccagatcgtgtccttctacttcaagctgttcaagaacttcaaggacgaccagagcatccagaaaagcgtggaaaccatcaaagaagatatgaacgtcaagttcttcaactccaacaagaagaagcgggacgacttcgagaagctgaccaactacagcgtgaccgacctgaacgtgcagagaaaggccatccacgagctgatccaagtgatggccgaactgtctcctgccgccaagaccggaaagcggaagagaagccagatgctgttcagaggcagacgggcctctcagtgattcg

SEQ ID NO: 25 - RNA, 587 nt, Homo sapiens
  mRNA construct for IFN alpha 16
gggagacgccaccauggcccugagcuucucucugcugauggcugugcuggugcugagcuacaagagcaucugcagccugggcugcgaccugccucagacacacucucugggaaacagacgggcccugauucugcuggcccagaugggcagaaucucccacuucagcugccugaaggacagauacgacuucggcuucccucaagagguguucgacggcaaccaguuccagaaggcccaggccaucucugccuuccacgagaugauccagcagaccuucaaccuguucagcaccaaggauagcagcgccgccugggaugagacacugcuggacaaguucuacaucgagcuguuccagcagcugaacgaccuggaagccugcgugacacaagaagugggcgucgaagagaucgcccugaugaacgaggauagcauccuggccgugcgcaaguacuuccagcggaucacccuguaccugaugggcaagaaguacagcccuugcgccugggaagucgugcgggccgaaaucaugagaagcuucagcuuuagcaccaaccugcagaagggccugagaagaaaggacugauucg

SEQ ID NO: 26 - RNA, 581 nt, Homo sapiens
  mRNA construct for IFN beta
gggagacgccaccaugaccaacaagugccugcugcagauugcccugcugcugugcuucagcacaacagcccugagcaugagcuacaaccugcugggcuuccugcagcggagcagcaacuuccagugccagaaacugcuguggcagcugaacggccggcuggaauacugccugaaggaccggaugaacuucgacauccccgaggaaaucaagcagcugcagcaguuccagaaagaggacgccgcucugaccaucuacgagaugcugcagaacaucuucgccaucuuccggcaggacagcagcuccacaggcuggaacgagacaaucguggaaaaucugcuggccaacguguaccaccagaucaaccaccugaaaaccgugcuggaagagaagcuggaaaaagaggacuucacccggggcaagcugaugagcagccugcaccugaagcgguacuacggcagaauccugcacuaccugaaggccaaagaguacagccacugcgccuggaccaucgugcgcguggaaauccugcggaacuucuacuucaucaaccggcugaccggcuaccugagaaacugauucg

SEQ ID NO: 27 - RNA, 518 nt, Homo sapiens
  mRNA construct for IFN gamma
gggagacgccaccaugaaguacaccagcuacauccuggccuuccagcugugcaucgugcugggaagccugggcugcuacugccaggauccuuacgugaaagaggccgagaaccugaagaaguacuuuaacgccggccacagcgacguggccgacaauggaacacuguuccugggcauccugaagaacuggaaagaggaaagcgaccggaagaucaugcagagccagaucguguccuucuacuucaagcuguucaagaacuucaaggacgaccagagcauccagaaaagcguggaaaccaucaaagaagauaugaacgucaaguucuucaacuccaacaagaagaagcgggacgacuucgagaagcugaccaacuacagcgugaccgaccugaacgugcagagaaaggccauccacgagcugauccaagugauggccgaacugucuccugccgccaagaccggaaagcggaagagaagccagaugcuguucagaggcagacgggccucucagugauucg

SEQ ID NO: 28 - DNA, 24 bp, Artificial Sequence
  M+24 F primer
agatgagtcttctaaccgaggtcg

SEQ ID NO: 29 - DNA, 24 bp, Artificial Sequence
  Rev-mod primer
tgcaaagacactttccagtctctg

SEQ ID NO: 30 - DNA, 20 bp, Artificial Sequence
  M+64 probe
tcaggccccctcaaagccga

SEQ ID NO: 31 - DNA, 20 bp, Artificial Sequence
  Fer_GAPDH FWD primer
caacggatttggccgtattg

SEQ ID NO: 32 - DNA, 23 bp, Artificial Sequence
  Fer_GAPDH REV primer
ctggaacatgtagaccatgtagt

SEQ ID NO: 33 - DNA, 27 bp, Artificial Sequence
  Fer_GAPDH PRB probe
agggtcattgatggcgacaatatccac

SEQ ID NO: 34 - DNA, 20 bp, Artificial Sequence
  SARS-CoV-2 N gene qPCR primer 1
aaattttggggaccaggaac

SEQ ID NO: 35 - DNA, 20 bp, Artificial Sequence
  SARS-CoV-2 N gene qPCR primer 2
tggcacctgtgtaggtcaac

SEQ ID NO: 36 - DNA, 20 bp, Artificial Sequence
  SARS-CoV-2 N gene qPCR probe
atgtcgcgcattggcatgga